European Patent Application EP 4 289 863 A1, published December 13, 2023. Title: BISPECIFIC ANTIBODY TARGETING IL-17A AND IL-36R AND APPLICATION THEREOF. Applicant: SHANGHAI HUAOTA BIOPHARMACEUTICAL CO., LTD. HUABO BIOPHARM (SHANGHAI) CO.,LTD. ZHEJIANG HUAHAI BIOPHARMACEUTICALS CO., LTD. The sequence listing filed with the application follows.

SEQUENCE LISTING (27 sequences)

SEQ ID NO: 1 - protein, 119 aa, Artificial Sequence
  heavy chain variable region of anti-IL-36R antibody
QVQLQQTGSVLVRPGTSVKLSCKASGYTFTSSWMHWAKQRPGQGLEWIGEIHPNSAKTNYNEKFKGKATLTVDTFSSTAYVDLSSLASEDSAVYYCARVDYGKPWFAYWGQGTLVTVSA

SEQ ID NO: 2 - protein, 108 aa, Artificial Sequence
  light chain variable region of anti-IL-36R antibody
QIVLTQSPTIMSASPGERVTMTCSASSSVSSSYLHWYQQKPGSSPKLWIYSTSNLASGVPARFSGSGSGTSYSLTINSMEAEDAATYYCQQFQSSPLTFGAGTKLGLK

SEQ ID NO: 3 - protein, 8 aa, Artificial Sequence
  HCDR1
GYTFTSSW

SEQ ID NO: 4 - protein, 8 aa, Artificial Sequence
  HCDR2
IHPNSAKT

SEQ ID NO: 5 - protein, 12 aa, Artificial Sequence
  HCDR3
ARVDYGKPWFAY

SEQ ID NO: 6 - protein, 7 aa, Artificial Sequence
  LCDR1
SSVSSSY

SEQ ID NO: 7 - protein, 3 aa, Artificial Sequence
  LCDR2
STS

SEQ ID NO: 8 - protein, 9 aa, Artificial Sequence
  LCDR3
QQFQSSPLT

SEQ ID NO: 9 - protein, 119 aa, Artificial Sequence
  VH
QVQLVQSGAEVKKPGASVKVSCKASGYTFTSSWMHWAKQAPGQGLEWIGEIHPNSAKTNYNQKFQGRVTMTRDTSISTAYMELSRLRSDDTAVYYCARVDYGKPWFAYWGQGTLVTVSS

SEQ ID NO: 10 - protein, 108 aa, Artificial Sequence
  VL
EIVLTQSPGTLSLSPGERATLSCSASSSVSSSYLHWYQQKPGQAPRLWIYSTSNRATGIPDRFSGSGSGTDFTLTISRLEPEDFATYYCQQFQSSPLTFGQGTKLEIK

SEQ ID NO: 11 - protein, 108 aa, Artificial Sequence
  VL
QIVLTQSPGTLSLSPGERATLSCRASSSVSSSYLHWYQQKPGQAPRLWIYSTSSRATGIPDRFSGSGSGTDFTLTISRLEPEDFATYYCQQFQSSPLTFGQGTKLEIK

SEQ ID NO: 12 - protein, 108 aa, Artificial Sequence
  VL
QIVLTQSPGTLSLSPGERATLSCRASSSVSSSYLHWYQQKPGQAPRLLIYSTSSRATGIPDRFSGSGSGTDFTLTISRLEPEDFATYYCQQFQSSPLTFGQGTKLEIK

SEQ ID NO: 13 - protein, 708 aa, Artificial Sequence
  H chian of bispecific antibody
QVQLVQSGSELKKPGASVKVSCKASEYIFTNYGMNWVKQAPGQGFEWMGWIDTNTGEPTYAQGFTGRFVFSLDTSVSTAYLQISSLKAEDTATYYCANYGWGYFDYWGQGTTVTVSSASTKGPSVFPLAPSSKSTSGGTAALGCLVKDYFPEPVTVSWNSGALTSGVHTFPAVLQSSGLYSLSSVVTVPSSSLGTQTYICNVNHKPSNTKVDKRVEPKSCDKTHTCPPCPAPEAAGGPSVFLFPPKPKDTLMISRTPEVTCVVVDVSHEDPEVKFNWYVDGVEVHNAKTKPREEQYNSTYRVVSVLTVLHQDWLNGKEYKCKVSNKALPAPIEKTISKAKGQPREPQVYTLPPSREEMTKNQVSLTCLVKGFYPSDIAVEWESNGQPENNYKTTPPVLDSDGSFFLYSKLTVDKSRWQQGNVFSCSVMHEALHNHYTQKSLSLSPGGGGGSGGGGSGGGGSGGGGSQIVLTQSPGTLSLSPGERATLSCRASSSVSSSYLHWYQQKPGQAPRLWIYSTSSRATGIPDRFSGSGSGTDFTLTISRLEPEDFATYYCQQFQSSPLTFGQGTKLEIKGGGGSGGGGSGGGGSQVQLVQSGAEVKKPGASVKVSCKASGYTFTSSWMHWAKQAPGQGLEWIGEIHPNSAKTNYNQKFQGRVTMTRDTSISTAYMELSRLRSDDTAVYYCARVDYGKPWFAYWGQGTLVTVSS

SEQ ID NO: 14 - protein, 708 aa, Artificial Sequence
  H chain of bispecific antibody
QVQLVQSGSELKKPGASVKVSCKASEYIFTNYGMNWVKQAPGQGFEWMGWIDTNTGEPTYAQGFTGRFVFSLDTSVSTAYLQISSLKAEDTATYYCANYGWGYFDYWGQGTTVTVSSASTKGPSVFPLAPSSKSTSGGTAALGCLVKDYFPEPVTVSWNSGALTSGVHTFPAVLQSSGLYSLSSVVTVPSSSLGTQTYICNVNHKPSNTKVDKRVEPKSCDKTHTCPPCPAPEAAGGPSVFLFPPKPKDTLMISRTPEVTCVVVDVSHEDPEVKFNWYVDGVEVHNAKTKPREEQYNSTYRVVSVLTVLHQDWLNGKEYKCKVSNKALPAPIEKTISKAKGQPREPQVYTLPPSREEMTKNQVSLTCLVKGFYPSDIAVEWESNGQPENNYKTTPPVLDSDGSFFLYSKLTVDKSRWQQGNVFSCSVMHEALHNHYTQKSLSLSPGGGGGSGGGGSGGGGSGGGGSQIVLTQSPGTLSLSPGERATLSCRASSSVSSSYLHWYQQKPGQAPRLWIYSTSSRATGIPDRFSGSGSGTDFTLTISRLEPEDFATYYCQQFQSSPLTFGCGTKLEIKGGGGSGGGGSGGGGSQVQLVQSGAEVKKPGASVKVSCKASGYTFTSSWMHWAKQAPGQCLEWIGEIHPNSAKTNYNQKFQGRVTMTRDTSISTAYMELSRLRSDDTAVYYCARVDYGKPWFAYWGQGTLVTVSS

SEQ ID NO: 15 - protein, 713 aa, Artificial Sequence
  H chain of bispecific antibody
QVQLVQSGSELKKPGASVKVSCKASEYIFTNYGMNWVKQAPGQGFEWMGWIDTNTGEPTYAQGFTGRFVFSLDTSVSTAYLQISSLKAEDTATYYCANYGWGYFDYWGQGTTVTVSSASTKGPSVFPLAPSSKSTSGGTAALGCLVKDYFPEPVTVSWNSGALTSGVHTFPAVLQSSGLYSLSSVVTVPSSSLGTQTYICNVNHKPSNTKVDKRVEPKSCDKTHTCPPCPAPEAAGGPSVFLFPPKPKDTLMISRTPEVTCVVVDVSHEDPEVKFNWYVDGVEVHNAKTKPREEQYNSTYRVVSVLTVLHQDWLNGKEYKCKVSNKALPAPIEKTISKAKGQPREPQVYTLPPSREEMTKNQVSLTCLVKGFYPSDIAVEWESNGQPENNYKTTPPVLDSDGSFFLYSKLTVDKSRWQQGNVFSCSVMHEALHNHYTQKSLSLSPGGGGGSGGGGSGGGGSGGGGSQIVLTQSPGTLSLSPGERATLSCRASSSVSSSYLHWYQQKPGQAPRLWIYSTSSRATGIPDRFSGSGSGTDFTLTISRLEPEDFATYYCQQFQSSPLTFGQGTKLEIKGGGGSGGGGSGGGGSGGGGSQVQLVQSGAEVKKPGASVKVSCKASGYTFTSSWMHWAKQAPGQGLEWIGEIHPNSAKTNYNQKFQGRVTMTRDTSISTAYMELSRLRSDDTAVYYCARVDYGKPWFAYWGQGTLVTVSS

SEQ ID NO: 16 - protein, 713 aa, Artificial Sequence
  H chain of bispecific antibody
QVQLVQSGSELKKPGASVKVSCKASEYIFTNYGMNWVKQAPGQGFEWMGWIDTNTGEPTYAQGFTGRFVFSLDTSVSTAYLQISSLKAEDTATYYCANYGWGYFDYWGQGTTVTVSSASTKGPSVFPLAPSSKSTSGGTAALGCLVKDYFPEPVTVSWNSGALTSGVHTFPAVLQSSGLYSLSSVVTVPSSSLGTQTYICNVNHKPSNTKVDKRVEPKSCDKTHTCPPCPAPEAAGGPSVFLFPPKPKDTLMISRTPEVTCVVVDVSHEDPEVKFNWYVDGVEVHNAKTKPREEQYNSTYRVVSVLTVLHQDWLNGKEYKCKVSNKALPAPIEKTISKAKGQPREPQVYTLPPSREEMTKNQVSLTCLVKGFYPSDIAVEWESNGQPENNYKTTPPVLDSDGSFFLYSKLTVDKSRWQQGNVFSCSVMHEALHNHYTQKSLSLSPGGGGGSGGGGSGGGGSGGGGSQIVLTQSPGTLSLSPGERATLSCRASSSVSSSYLHWYQQKPGQAPRLWIYSTSSRATGIPDRFSGSGSGTDFTLTISRLEPEDFATYYCQQFQSSPLTFGCGTKLEIKGGGGSGGGGSGGGGSGGGGSQVQLVQSGAEVKKPGASVKVSCKASGYTFTSSWMHWAKQAPGQCLEWIGEIHPNSAKTNYNQKFQGRVTMTRDTSISTAYMELSRLRSDDTAVYYCARVDYGKPWFAYWGQGTLVTVSS

SEQ ID NO: 17 - protein, 718 aa, Artificial Sequence
  H chain of bispecific antibody
QVQLVQSGSELKKPGASVKVSCKASEYIFTNYGMNWVKQAPGQGFEWMGWIDTNTGEPTYAQGFTGRFVFSLDTSVSTAYLQISSLKAEDTATYYCANYGWGYFDYWGQGTTVTVSSASTKGPSVFPLAPSSKSTSGGTAALGCLVKDYFPEPVTVSWNSGALTSGVHTFPAVLQSSGLYSLSSVVTVPSSSLGTQTYICNVNHKPSNTKVDKRVEPKSCDKTHTCPPCPAPEAAGGPSVFLFPPKPKDTLMISRTPEVTCVVVDVSHEDPEVKFNWYVDGVEVHNAKTKPREEQYNSTYRVVSVLTVLHQDWLNGKEYKCKVSNKALPAPIEKTISKAKGQPREPQVYTLPPSREEMTKNQVSLTCLVKGFYPSDIAVEWESNGQPENNYKTTPPVLDSDGSFFLYSKLTVDKSRWQQGNVFSCSVMHEALHNHYTQKSLSLSPGGGGGSGGGGSGGGGSGGGGSQIVLTQSPGTLSLSPGERATLSCRASSSVSSSYLHWYQQKPGQAPRLWIYSTSSRATGIPDRFSGSGSGTDFTLTISRLEPEDFATYYCQQFQSSPLTFGQGTKLEIKGGGGSGGGGSGGGGSGGGGSGGGGSQVQLVQSGAEVKKPGASVKVSCKASGYTFTSSWMHWAKQAPGQGLEWIGEIHPNSAKTNYNQKFQGRVTMTRDTSISTAYMELSRLRSDDTAVYYCARVDYGKPWFAYWGQGTLVTVSS

SEQ ID NO: 18 - protein, 718 aa, Artificial Sequence
  H chain of bispecific antibody
QVQLVQSGSELKKPGASVKVSCKASEYIFTNYGMNWVKQAPGQGFEWMGWIDTNTGEPTYAQGFTGRFVFSLDTSVSTAYLQISSLKAEDTATYYCANYGWGYFDYWGQGTTVTVSSASTKGPSVFPLAPSSKSTSGGTAALGCLVKDYFPEPVTVSWNSGALTSGVHTFPAVLQSSGLYSLSSVVTVPSSSLGTQTYICNVNHKPSNTKVDKRVEPKSCDKTHTCPPCPAPEAAGGPSVFLFPPKPKDTLMISRTPEVTCVVVDVSHEDPEVKFNWYVDGVEVHNAKTKPREEQYNSTYRVVSVLTVLHQDWLNGKEYKCKVSNKALPAPIEKTISKAKGQPREPQVYTLPPSREEMTKNQVSLTCLVKGFYPSDIAVEWESNGQPENNYKTTPPVLDSDGSFFLYSKLTVDKSRWQQGNVFSCSVMHEALHNHYTQKSLSLSPGGGGGSGGGGSGGGGSGGGGSQIVLTQSPGTLSLSPGERATLSCRASSSVSSSYLHWYQQKPGQAPRLWIYSTSSRATGIPDRFSGSGSGTDFTLTISRLEPEDFATYYCQQFQSSPLTFGCGTKLEIKGGGGSGGGGSGGGGSGGGGSGGGGSQVQLVQSGAEVKKPGASVKVSCKASGYTFTSSWMHWAKQAPGQCLEWIGEIHPNSAKTNYNQKFQGRVTMTRDTSISTAYMELSRLRSDDTAVYYCARVDYGKPWFAYWGQGTLVTVSS

SEQ ID NO: 19 - protein, 219 aa, Artificial Sequence
  L chain of bispecific antibody
DVVMTQTPPSLPVNPGEPASISCRSSQSLVHSNGYTYLHWYLQKPGQSPQLLIYKVSNHLSGVPDRFSGSGSGTDFTLKISWVEAEDVGVYFCSQSTHVPYTFGGGTKLEIKRTVAAPSVFIFPPSDEQLKSGTASVVCLLNNFYPREAKVQWKVDNALQSGNSQESVTEQDSKDSTYSLSSTLTLSKADYEKHKVYACEVTHQGLSSPVTKSFNRGEC

SEQ ID NO: 20 - protein, 7 aa, Artificial Sequence
  HCDR1 of anti-IL-17A antibody
EYIFTNY

SEQ ID NO: 21 - protein, 6 aa, Artificial Sequence
  HCDR2 of anti-IL-17A antibody
DTNTGE

SEQ ID NO: 22 - protein, 10 aa, Artificial Sequence
  HCDR3 of anti-IL-17A antibody
ANYGWGYFDY

SEQ ID NO: 23 - protein, 11 aa, Artificial Sequence
  LCDR1 of anti-IL-17A antibody
QSLVHSNGYTY

SEQ ID NO: 24 - protein, 3 aa, Artificial Sequence
  LCDR2 of anti-IL-17A antibody
KVS

SEQ ID NO: 25 - protein, 9 aa, Artificial Sequence
  LCDR3 of anti-IL-17A antibody
SQSTHVPYT

SEQ ID NO: 26 - protein, 117 aa, Artificial Sequence
  VH of scFV of anti-IL-17A antibody
QVQLVQSGSELKKPGASVKVSCKASEYIFTNYGMNWVKQAPGQGFEWMGWIDTNTGEPTYAQGFTGRFVFSLDTSVSTAYLQISSLKAEDTATYYCANYGWGYFDYWGQGTTVTVSS

SEQ ID NO: 27 - protein, 112 aa, Artificial Sequence
  VL of scFV of anti-IL-17A antibody
DVVMTQTPPSLPVNPGEPASISCRSSQSLVHSNGYTYLHWYLQKPGQSPQLLIYKVSNHLSGVPDRFSGSGSGTDFTLKISWVEAEDVGVYFCSQSTHVPYTFGGGTKLEIK